European Patent Specification EP 3 234 120 B1, published September 3, 2025. Title: Cytotoxic Molecules Responsive to Intracellular Ligands for Selective T Cell Mediated Killing. Applicant: Chen, Yvonne Yu-Hsuan Ho, Patrick. The sequence listing filed with the application follows.

SEQUENCE LISTING (10 sequences)

SEQ ID NO: 1 - protein, 227 aa, Homo sapiens
IIGGHEAKPHSRPYMAYLMIWDQKSLKRCGGFLIQDDFVLTAAHCWGSSINVTLGAHNIKEQEPTQQFIPVKRPIPHPAYNPKNFSNDIMLLQLERKAKRTRAVQPLRLPSNKAQVKPGQTCSVAGWGQTAPLGKHSHTLQEVKMTVQEDRKCESDLRHYYDSTIELCVGDPEIKKTSFKGDSGGPLVCNKVAQGIVSYGRNNGMPPRACTKVSSFVHWIKKTMKRY

SEQ ID NO: 2 - protein, 173 aa, Homo sapiens
IIGGHEAKPHSRPYMAYLMIWDQKSLKRCGGFLIQDDFVLTAAHCWGSSINVTLGAHNIKEQEPTQQFIPVKRPIPHPAYNPKNFSNDIMLLQLERKAKRTRAVQPLRLPSNKAQVKPGQTCSVAGWGQTAPLGKHSHTLQEVKMTVQEDRKCESDLRHYYDSTIELCVGDPE

SEQ ID NO: 3 - protein, 54 aa, Homo sapiens
IKKTSFKGDSGGPLVCNKVAQGIVSYGRNNGMPPRACTKVSSFVHWIKKTMKRY

SEQ ID NO: 4 - protein, 357 aa, Homo sapiens
AATMETDTLLLWVLLLWVPGSTGHHHHHHDDDDKSDQEAKPSTEDLGDKKEGEYIKLKVIGQDSSEIHFKVKMTTHLKKLKESYCQRQGVPMNSLRFLFEGQRIADNHTPKELGMEEEDVIEVYQEQTGGIIGGHEAKPHSRPYMAYLMIWDQKSLKRCGGFLIQDDFVLTAAHCWGSSINVTLGAHNIKEQEPTQQFIPVKRPIPHPAYNPKNFSNDIMLLQLERKAKRTRAVQPLRLPSNKAQVKPGQTCSVAGWGQTAPLGKHSHTLQEVKMTVQEDRKCESDLRHYYDSTIELCVGDPEIKKTSFKGDSGGPLVCNKVAQGIVSYGRNNGMPPRACTKVSSFVHWIKKTMKRY

SEQ ID NO: 5 - protein, 20 aa, Homo sapiens
METDTLLLWVLLLWVPGSTG

SEQ ID NO: 6 - protein, 96 aa, Homo sapiens
SDQEAKPSTEDLGDKKEGEYIKLKVIGQDSSEIHFKVKMTTHLKKLKESYCQRQGVPMNSLRFLFEGQRIADNHTPKELGMEEEDVIEVYQEQTGG

SEQ ID NO: 7 - protein, 26 aa, Homo sapiens
GSSGSGSTGSGSSGTGSSGTSGTGTS

SEQ ID NO: 8 - protein, 9 aa, Homo sapiens
GSSTGGGGS

SEQ ID NO: 9 - protein, 14 aa, Homo sapiens
GSSGSGSSGSGSSG

SEQ ID NO: 10 - protein, 5 aa, Homo sapiens
GGGGS